European Patent Specification EP 3 172 232 B1, published December 27, 2023. Title: SITE DIRECTED MUTAGENESIS OF TREM-1 ANTIBODIES. Applicant: Novo Nordisk A/S. The sequence listing filed with the application follows.

SEQUENCE LISTING (19 sequences)

SEQ ID NO: 1 - protein, 234 aa, Homo Sapiens
MRKTRLWGLLWMLFVSELRAATKLTEEKYELKEGQTLDVKCDYTLEKFASSQKAWQIIRDGEMPKTLACTERPSKNSHPVQVGRIILEDYHDHGLLRVRMVNLQVEDSGLYQCVIYQPPKEPHMLFDRIRLVVTKGFSGTPGSNENSTQNVYKIPPTTTKALCPLYTSPRTVTQAPPKSTADVSTPDSEINLTNVTDIIRVPVFNIVILLAGGFLSKSLVFSVLFAVTLRSFVP

SEQ ID NO: 2 - protein, 448 aa, Artificial Sequence
  heavy chain of a humanised TREM-1 antibody
EVQLVESGGGLVQPGGSLKLSCAASGFTFSTYAMHWVRQASGKGLEWVGRIRTKSSNYATYYAASVKGRFTISRDDSKNTAYLQMNSLKTEDTAVYYCTRDMGIRRQFAYWGQGTLVTVSSASTKGPSVFPLAPCSRSTSESTAALGCLVKDYFPEPVTVSWNSGALTSGVHTFPAVLQSSGLYSLSSVVTVPSSSLGTKTYTCNVDHKPSNTKVDKRVESKYGPPCPPCPAPEFLGGPSVFLFPPKPKDTLMISRTPEVTCVVVDVSQEDPEVQFNWYVDGVEVHNAKTKPREEQFNSTYRVVSVLTVLHQDWLNGKEYKCKVSNKGLPSSIEKTISKAKGQPREPQVYTLPPSQEEMTKNQVSLTCLVKGFYPSDIAVEWESNGQPENNYKTTPPVLDSDGSFFLYSRLTVDKSRWQEGNVFSCSVMHEALHNHYTQKSLSLSLGK

SEQ ID NO: 3 - protein, 218 aa, Artificial Sequence
  CHAIN (1)..(218): light chain of a humanised TREM-1 antibody
DIVLTQSPDSLAVSLGERATINCRASESVDTFDYSFLHWYQQKPGQPPKLLIYRASNLESGVPDRFSGSGSGTDFTLTISSLQAEDVAVYYCQQSNEDPYTFGQGTKLEIKRTVAAPSVFIFPPSDEQLKSGTASVVCLLNNFYPREAKVQWKVDNALQSGNSQESVTEQDSKDSTYSLSSTLTLSKADYEKHKVYACEVTHQGLSSPVTKSFNRGEC

SEQ ID NO: 4 - protein, 218 aa, Artificial Sequence
  light chain of a humanised TREM-1 antibody
DIVLTQSPDSLAVSLGERATINCRASQSVDTFDYSFLHWYQQKPGQPPKLLIYRASNLESGVPDRFSGSGSGTDFTLTISSLQAEDVAVYYCQQSNSDPYTFGQGTKLEIKRTVAAPSVFIFPPSDEQLKSGTASVVCLLNNFYPREAKVQWKVDNALQSGNSQESVTEQDSKDSTYSLSSTLTLSKADYEKHKVYACEVTHQGLSSPVTKSFNRGEC

SEQ ID NO: 5 - protein, 218 aa, Artificial Sequence
DIVLTQSPDSLAVSLGERATINCRASQSVDTFDYSFLHWYQQKPGQPPKLLIYRASNLESGVPDRFSGSGSGTDFTLTISSLQAEDVAVYYCQQSNQDPYTFGQGTKLEIKRTVAAPSVFIFPPSDEQLKSGTASVVCLLNNFYPREAKVQWKVDNALQSGNSQESVTEQDSKDSTYSLSSTLTLSKADYEKHKVYACEVTHQGLSSPVTKSFNRGEC

SEQ ID NO: 6 - protein, 218 aa, Artificial Sequence
  light chain of a humanised TREM-1 antibody
DIVLTQSPDSLAVSLGERATINCRASESVDTFDYSFLHWYQQKPGQPPKLLIYRASNLESGVPDRFSGSGSGTDFTLTISSLQAEDVAVYYCQQSNSDPYTFGQGTKLEIKRTVAAPSVFIFPPSDEQLKSGTASVVCLLNNFYPREAKVQWKVDNALQSGNSQESVTEQDSKDSTYSLSSTLTLSKADYEKHKVYACEVTHQGLSSPVTKSFNRGEC

SEQ ID NO: 7 - protein, 218 aa, Artificial Sequence
  light chain of a humanised TREM-1 antibody
DIVLTQSPDSLAVSLGERATINCRASESVDTFDYSFLHWYQQKPGQPPKLLIYRASNLESGVPDRFSGSGSGTDFTLTISSLQAEDVAVYYCQQSNQDPYTFGQGTKLEIKRTVAAPSVFIFPPSDEQLKSGTASVVCLLNNFYPREAKVQWKVDNALQSGNSQESVTEQDSKDSTYSLSSTLTLSKADYEKHKVYACEVTHQGLSSPVTKSFNRGEC

SEQ ID NO: 8 - protein, 218 aa, Artificial Sequence
  light chain of a humanised TREM-1 antibody
DIVLTQSPDSLAVSLGERATINCRASQSVDTFDYSFLHWYQQKPGQPPKLLIYRASNLESGVPDRFSGSGSGTDFTLTISSLQAEDVAVYYCQQSNEDPYTFGQGTKLEIKRTVAAPSVFIFPPSDEQLKSGTASVVCLLNNFYPREAKVQWKVDNALQSGNSQESVTEQDSKDSTYSLSSTLTLSKADYEKHKVYACEVTHQGLSSPVTKSFNRGEC

SEQ ID NO: 9 - protein, 218 aa, Artificial Sequence
  light chain of a humanised TREM-1 antibody
DIVLTQSPDSLAVSLGERATINCRASESVDTADYSFLHWYQQKPGQPPKLLIYRASNLESGVPDRFSGSGSGTDFTLTISSLQAEDVAVYYCQQSNEDPYTFGQGTKLEIKRTVAAPSVFIFPPSDEQLKSGTASVVCLLNNFYPREAKVQWKVDNALQSGNSQESVTEQDSKDSTYSLSSTLTLSKADYEKHKVYACEVTHQGLSSPVTKSFNRGEC

SEQ ID NO: 10 - protein, 218 aa, Artificial Sequence
  light chain of a humanised TREM-1 antibody
DIVLTQSPDSLAVSLGERATINCRASESVDTSDYSFLHWYQQKPGQPPKLLIYRASNLESGVPDRFSGSGSGTDFTLTISSLQAEDVAVYYCQQSNEDPYTFGQGTKLEIKRTVAAPSVFIFPPSDEQLKSGTASVVCLLNNFYPREAKVQWKVDNALQSGNSQESVTEQDSKDSTYSLSSTLTLSKADYEKHKVYACEVTHQGLSSPVTKSFNRGEC

SEQ ID NO: 11 - protein, 448 aa, Artificial Sequence
  heavy chain of a humanised TREM-1 antibody
EVQLVESGGGLVQPGGSLKLSCAASGFTFSTYAMHWVRQASGKGLEWVGRIRTKSSNYYTYYAASVKGRFTISRDDSKNTAYLQMNSLKTEDTAVYYCTRDMGIRRQFAYWGQGTLVTVSSASTKGPSVFPLAPCSRSTSESTAALGCLVKDYFPEPVTVSWNSGALTSGVHTFPAVLQSSGLYSLSSVVTVPSSSLGTKTYTCNVDHKPSNTKVDKRVESKYGPPCPPCPAPEFLGGPSVFLFPPKPKDTLMISRTPEVTCVVVDVSQEDPEVQFNWYVDGVEVHNAKTKPREEQFNSTYRVVSVLTVLHQDWLNGKEYKCKVSNKGLPSSIEKTISKAKGQPREPQVYTLPPSQEEMTKNQVSLTCLVKGFYPSDIAVEWESNGQPENNYKTTPPVLDSDGSFFLYSRLTVDKSRWQEGNVFSCSVMHEALHNHYTQKSLSLSLGK

SEQ ID NO: 12 - protein, 448 aa, Artificial Sequence
  heavy chain of a humanised TREM-1 antibody
EVQLVESGGGLVQPGGSLKLSCAASGFTFSTYAMHWVRQASGKGLEWVGRIRTKSSSYATYYAASVKGRFTISRDDSKNTAYLQMNSLKTEDTAVYYCTRDMGIRRQFAYWGQGTLVTVSSASTKGPSVFPLAPCSRSTSESTAALGCLVKDYFPEPVTVSWNSGALTSGVHTFPAVLQSSGLYSLSSVVTVPSSSLGTKTYTCNVDHKPSNTKVDKRVESKYGPPCPPCPAPEFLGGPSVFLFPPKPKDTLMISRTPEVTCVVVDVSQEDPEVQFNWYVDGVEVHNAKTKPREEQFNSTYRVVSVLTVLHQDWLNGKEYKCKVSNKGLPSSIEKTISKAKGQPREPQVYTLPPSQEEMTKNQVSLTCLVKGFYPSDIAVEWESNGQPENNYKTTPPVLDSDGSFFLYSRLTVDKSRWQEGNVFSCSVMHEALHNHYTQKSLSLSLGK

SEQ ID NO: 13 - protein, 448 aa, Artificial Sequence
  heavy chain of a humanised TREM-1 antibody
EVQLVESGGGLVQPGGSLKLSCAASGFTFSTYAMHWVRQASGKGLEWVGRIRTKSSSYYTYYAASVKGRFTISRDDSKNTAYLQMNSLKTEDTAVYYCTRDMGIRRQFAYWGQGTLVTVSSASTKGPSVFPLAPCSRSTSESTAALGCLVKDYFPEPVTVSWNSGALTSGVHTFPAVLQSSGLYSLSSVVTVPSSSLGTKTYTCNVDHKPSNTKVDKRVESKYGPPCPPCPAPEFLGGPSVFLFPPKPKDTLMISRTPEVTCVVVDVSQEDPEVQFNWYVDGVEVHNAKTKPREEQFNSTYRVVSVLTVLHQDWLNGKEYKCKVSNKGLPSSIEKTISKAKGQPREPQVYTLPPSQEEMTKNQVSLTCLVKGFYPSDIAVEWESNGQPENNYKTTPPVLDSDGSFFLYSRLTVDKSRWQEGNVFSCSVMHEALHNHYTQKSLSLSLGK

SEQ ID NO: 14 - protein, 218 aa, Artificial Sequence
  light chain of a humanised TREM-1 antibody
DIVLTQSPDSLAVSLGERATINCRASQSVDTADYSFLHWYQQKPGQPPKLLIYRASNLESGVPDRFSGSGSGTDFTLTISSLQAEDVAVYYCQQSNQDPYTFGQGTKLEIKRTVAAPSVFIFPPSDEQLKSGTASVVCLLNNFYPREAKVQWKVDNALQSGNSQESVTEQDSKDSTYSLSSTLTLSKADYEKHKVYACEVTHQGLSSPVTKSFNRGEC

SEQ ID NO: 15 - protein, 448 aa, Artificial Sequence; identical to SEQ ID NO: 11
  heavy chain of a humanised TREM-1 antibody

SEQ ID NO: 16 - protein, 448 aa, Artificial Sequence; identical to SEQ ID NO: 11
  heavy chain of a humanised TREM-1 antibody

SEQ ID NO: 17 - protein, 233 aa, Macaca fascicularis
MRKTRLWGLLWMLFVSELRATTELTEEKYEYKEGQTLEVKCDYALEKYANSRKAWQKMEGKMPKILAKTERPSENSHPVQVGRITLEDYPDHGLLQVQMTNLQVEDSGLYQCVIYQHPKESHVLFNPICLVVTKGSSGTPGSSENSTQNVYRTPSTTAKALGPRYTSPRTVTQAPPESTVVVSTPGSEINLTNVTDIIRVPVFNIVIIVAGGFLSKSLVFSVLFAVTLRSFGP

SEQ ID NO: 18 - protein, 219 aa, artificial sequence
  Expression construct for crystallization
EVQLVESGGGLVQPGGSLKLSCAASGFTFSTYAMHWVRQASGKGLEWVGRIRTKSSNYATYYAASVKGRFTISRDDSKNTAYLQMNSLKTEDTAVYYCTRDMGIRRQFAYWGQGTLVTVSSASTKGPSVFPLAPCSRSTSESTAALGCLVKDYFPEPVTVSWNSGALTSGVHTFPAVLQSSGLYSLSSVVTVPSSSLGTKTYTCNVDHKPSNTKVDKRV

SEQ ID NO: 19 - protein, 218 aa, artificial sequence; identical to SEQ ID NO: 3
  Expression construct for crystallization